European Patent Specification EP 3 532 090 B1, published March 25, 2026. Title: ENDOGLYCOSIDASE MUTANTS FOR GLYCOPROTEIN REMODELING AND METHODS OF USING IT. Applicant: CHO Pharma Inc. Academia Sinica Nan-Horng Lin. The sequence listing filed with the application follows.

SEQUENCE LISTING (19 sequences)

SEQ ID NO: 1 - protein, 842 aa, Streptococcus pyogenes
MDKHLLVKRTLGCVCAATLMGAALATHHDSLNTVKAEEKTVQTGKTDQQVGAKLVQEIREGKRGPLYAGYFRTWHDRASTGIDGKQQHPENTMAEVPKEVDILFVFHDHTASDSPFWSELKDSYVHKLHQQGTALVQTIGVNELNGRTGLSKDYPDTPEGNKALAAAIVKAFVTDRGVDGLDIDIEHEFTNKRTPEEDARALNVFKEIAQLIGKNGSDKSKLLIMDTTLSVENNPIFKGIAEDLDYLLRQYYGSQGGEAEVDTINSDWNQYQNYIDASQFMIGFSFFEESASKGNLWFDVNEYDPNNPEKGKDIEGTRAKKYAEWQPSTGGLKAGIFSYAIDRDGVAHVPSTYKNRTSTNLQRHEVDNISHTDYTVSRKLKTLMTEDKRYDVIDQKDIPDPALREQIIQQVGQYKGDLERYNKTLVLTGDKIQNLKGLEKLSKLQKLELRQLSNVKEITPELLPESMKKDAELVMVGMTGLEKLNLSGLNRQTLDGIDVNSITHLTSFDISHNSLDLSEKSEDRKLLMTLMEQVSNHQKITVKNTAFENQKPKGYYPQTYDTKEGHYDVDNAEHDILTDFVFGTVTKRNTFIGDEEAFAIYKEGAVDGRQYVSKDYTYEAFRKDYKGYKVHLTASNLGETVTSKVTATTDETYLVDVSDGEKVVHHMKLNIGSGAIMMENLAKGAKVIGTSGDFEQAKKIFDGEKSDRFFTWGQTNWIAFDLGEINLAKEWRLFNAETNTEIKTDSSLNVAKGRLQILKDTTIDLEKMDIKNRKEYLSNDENWTDVAQMDDAKAIFNSKLSNVLSRYWRFCVDGGASSYYPQYTELQILGQRLSNDVANTLD

SEQ ID NO: 2 - protein, 842 aa, Artificial Sequence
  Synthetic
MDKHLLVKRTLGCVCAATLMGAALATHHDSLNTVKAEEKTVQTGKTDQQVGAKLVQEIREGKRGPLYAGYFRTWHDRASTGIDGKQQHPENTMAEVPKEVDILFVFHDHTASDSPFWSELKDSYVHKLHQQGTALVQTIGVNELNGRTGLSKDYPDTPEGNKALAAAIVKAFVTDRGVDGLQIDIEHEFTNKRTPEEDARALNVFKEIAQLIGKNGSDKSKLLIMDTTLSVENNPIFKGIAEDLDYLLRQYYGSQGGEAEVDTINSDWNQYQNYIDASQFMIGFSFFEESASKGNLWFDVNEYDPNNPEKGKDIEGTRAKKYAEWQPSTGGLKAGIFSYAIDRDGVAHVPSTYKNRTSTNLQRHEVDNISHTDYTVSRKLKTLMTEDKRYDVIDQKDIPDPALREQIIQQVGQYKGDLERYNKTLVLTGDKIQNLKGLEKLSKLQKLELRQLSNVKEITPELLPESMKKDAELVMVGMTGLEKLNLSGLNRQTLDGIDVNSITHLTSFDISHNSLDLSEKSEDRKLLMTLMEQVSNHQKITVKNTAFENQKPKGYYPQTYDTKEGHYDVDNAEHDILTDFVFGTVTKRNTFIGDEEAFAIYKEGAVDGRQYVSKDYTYEAFRKDYKGYKVHLTASNLGETVTSKVTATTDETYLVDVSDGEKVVHHMKLNIGSGAIMMENLAKGAKVIGTSGDFEQAKKIFDGEKSDRFFTWGQTNWIAFDLGEINLAKEWRLFNAETNTEIKTDSSLNVAKGRLQILKDTTIDLEKMDIKNRKEYLSNDENWTDVAQMDDAKAIFNSKLSNVLSRYWRFCVDGGASSYYPQYTELQILGQRLSNDVANTLD

SEQ ID NO: 3 - protein, 842 aa, Artificial Sequence
  Synthetic
MDKHLLVKRTLGCVCAATLMGAALATHHDSLNTVKAEEKTVQTGKTDQQVGAKLVQEIREGKRGPLYAGYFRTWHDRASTGIDGKQQHPENTMAEVPKEVDILFVFHDHTASDSPFWSELKDSYVHKLHQQGTALVQTIGVNELNGRTGLSKDYPDTPEGNKALAAAIVKAFVTDRGVDGLDIDIEHEFTNKRTPEEDARALNVFKEIAQLIGKNGSDKSKLLIMQTTLSVENNPIFKGIAEDLDYLLRQYYGSQGGEAEVDTINSDWNQYQNYIDASQFMIGFSFFEESASKGNLWFDVNEYDPNNPEKGKDIEGTRAKKYAEWQPSTGGLKAGIFSYAIDRDGVAHVPSTYKNRTSTNLQRHEVDNISHTDYTVSRKLKTLMTEDKRYDVIDQKDIPDPALREQIIQQVGQYKGDLERYNKTLVLTGDKIQNLKGLEKLSKLQKLELRQLSNVKEITPELLPESMKKDAELVMVGMTGLEKLNLSGLNRQTLDGIDVNSITHLTSFDISHNSLDLSEKSEDRKLLMTLMEQVSNHQKITVKNTAFENQKPKGYYPQTYDTKEGHYDVDNAEHDILTDFVFGTVTKRNTFIGDEEAFAIYKEGAVDGRQYVSKDYTYEAFRKDYKGYKVHLTASNLGETVTSKVTATTDETYLVDVSDGEKVVHHMKLNIGSGAIMMENLAKGAKVIGTSGDFEQAKKIFDGEKSDRFFTWGQTNWIAFDLGEINLAKEWRLFNAETNTEIKTDSSLNVAKGRLQILKDTTIDLEKMDIKNRKEYLSNDENWTDVAQMDDAKAIFNSKLSNVLSRYWRFCVDGGASSYYPQYTELQILGQRLSNDVANTLD

SEQ ID NO: 4 - protein, 842 aa, Artificial Sequence
  Synthetic
MDKHLLVKRTLGCVCAATLMGAALATHHDSLNTVKAEEKTVQTGKTDQQVGAKLVQEIREGKRGPLYAGYFRTWHDRASTGIDGKQQHPENTMAEVPKEVDILFVFHDHTASDSPFWSELKDSYVHKLHQQGTALVQTIGVNELNGRTGLSKDYPDTPEGNKALAAAIVKAFVTDRGVDGLDIDIEHEFTNKRTPEEDARALNVFKEIAQLIGKNGSDKSKLLIMDQTLSVENNPIFKGIAEDLDYLLRQYYGSQGGEAEVDTINSDWNQYQNYIDASQFMIGFSFFEESASKGNLWFDVNEYDPNNPEKGKDIEGTRAKKYAEWQPSTGGLKAGIFSYAIDRDGVAHVPSTYKNRTSTNLQRHEVDNISHTDYTVSRKLKTLMTEDKRYDVIDQKDIPDPALREQIIQQVGQYKGDLERYNKTLVLTGDKIQNLKGLEKLSKLQKLELRQLSNVKEITPELLPESMKKDAELVMVGMTGLEKLNLSGLNRQTLDGIDVNSITHLTSFDISHNSLDLSEKSEDRKLLMTLMEQVSNHQKITVKNTAFENQKPKGYYPQTYDTKEGHYDVDNAEHDILTDFVFGTVTKRNTFIGDEEAFAIYKEGAVDGRQYVSKDYTYEAFRKDYKGYKVHLTASNLGETVTSKVTATTDETYLVDVSDGEKVVHHMKLNIGSGAIMMENLAKGAKVIGTSGDFEQAKKIFDGEKSDRFFTWGQTNWIAFDLGEINLAKEWRLFNAETNTEIKTDSSLNVAKGRLQILKDTTIDLEKMDIKNRKEYLSNDENWTDVAQMDDAKAIFNSKLSNVLSRYWRFCVDGGASSYYPQYTELQILGQRLSNDVANTLD

SEQ ID NO: 5 - protein, 842 aa, Artificial Sequence
  Synthetic
MDKHLLVKRTLGCVCAATLMGAALATHHDSLNTVKAEEKTVQTGKTDQQVGAKLVQEIREGKRGPLYAGYFRTWHDRASTGIDGKQQHPENTMAEVPKEVDILFVFHDHTASDSPFWSELKDSYVHKLHQQGTALVQTIGVNELNGRTGLSKDYPDTPEGNKALAAAIVKAFVTDRGVDGLDIDIEHEFTNKRTPEEDARALNVFKEIAQLIGKNGSDKSKLLIMDTQLSVENNPIFKGIAEDLDYLLRQYYGSQGGEAEVDTINSDWNQYQNYIDASQFMIGFSFFEESASKGNLWFDVNEYDPNNPEKGKDIEGTRAKKYAEWQPSTGGLKAGIFSYAIDRDGVAHVPSTYKNRTSTNLQRHEVDNISHTDYTVSRKLKTLMTEDKRYDVIDQKDIPDPALREQIIQQVGQYKGDLERYNKTLVLTGDKIQNLKGLEKLSKLQKLELRQLSNVKEITPELLPESMKKDAELVMVGMTGLEKLNLSGLNRQTLDGIDVNSITHLTSFDISHNSLDLSEKSEDRKLLMTLMEQVSNHQKITVKNTAFENQKPKGYYPQTYDTKEGHYDVDNAEHDILTDFVFGTVTKRNTFIGDEEAFAIYKEGAVDGRQYVSKDYTYEAFRKDYKGYKVHLTASNLGETVTSKVTATTDETYLVDVSDGEKVVHHMKLNIGSGAIMMENLAKGAKVIGTSGDFEQAKKIFDGEKSDRFFTWGQTNWIAFDLGEINLAKEWRLFNAETNTEIKTDSSLNVAKGRLQILKDTTIDLEKMDIKNRKEYLSNDENWTDVAQMDDAKAIFNSKLSNVLSRYWRFCVDGGASSYYPQYTELQILGQRLSNDVANTLD

SEQ ID NO: 6 - protein, 842 aa, Artificial Sequence
  Synthetic
MDKHLLVKRTLGCVCAATLMGAALATHHDSLNTVKAEEKTVQTGKTDQQVGAKLVQEIREGKRGPLYAGYFRTWHDRASTGIDGKQQHPENTMAEVPKEVDILFVFHDHTASDSPFWSELKDSYVHKLHQQGTALVQDIGVNELNGRTGLSKDYPDTPEGNKALAAAIVKAFVTDRGVDGLDIDIEHEFTNKRTPEEDARALNVFKEIAQLIGKNGSDKSKLLIMDTTLSVENNPIFKGIAEDLDYLLRQYYGSQGGEAEVDTINSDWNQYQNYIDASQFMIGFSFFEESASKGNLWFDVNEYDPNNPEKGKDIEGTRAKKYAEWQPSTGGLKAGIFSYAIDRDGVAHVPSTYKNRTSTNLQRHEVDNISHTDYTVSRKLKTLMTEDKRYDVIDQKDIPDPALREQIIQQVGQYKGDLERYNKTLVLTGDKIQNLKGLEKLSKLQKLELRQLSNVKEITPELLPESMKKDAELVMVGMTGLEKLNLSGLNRQTLDGIDVNSITHLTSFDISHNSLDLSEKSEDRKLLMTLMEQVSNHQKITVKNTAFENQKPKGYYPQTYDTKEGHYDVDNAEHDILTDFVFGTVTKRNTFIGDEEAFAIYKEGAVDGRQYVSKDYTYEAFRKDYKGYKVHLTASNLGETVTSKVTATTDETYLVDVSDGEKVVHHMKLNIGSGAIMMENLAKGAKVIGTSGDFEQAKKIFDGEKSDRFFTWGQTNWIAFDLGEINLAKEWRLFNAETNTEIKTDSSLNVAKGRLQILKDTTIDLEKMDIKNRKEYLSNDENWTDVAQMDDAKAIFNSKLSNVLSRYWRFCVDGGASSYYPQYTELQILGQRLSNDVANTLD

SEQ ID NO: 7 - protein, 842 aa, Artificial Sequence
  Synthetic
MDKHLLVKRTLGCVCAATLMGAALATHHDSLNTVKAEEKTVQTGKTDQQVGAKLVQEIREGKRGPLYAGYFRTWHDRASTGIDGKQQHPENTMAEVPKEVDILFVFHDHTASDSPFWSELKDSYVHKLHQQGTALVQEIGVNELNGRTGLSKDYPDTPEGNKALAAAIVKAFVTDRGVDGLDIDIEHEFTNKRTPEEDARALNVFKEIAQLIGKNGSDKSKLLIMDTTLSVENNPIFKGIAEDLDYLLRQYYGSQGGEAEVDTINSDWNQYQNYIDASQFMIGFSFFEESASKGNLWFDVNEYDPNNPEKGKDIEGTRAKKYAEWQPSTGGLKAGIFSYAIDRDGVAHVPSTYKNRTSTNLQRHEVDNISHTDYTVSRKLKTLMTEDKRYDVIDQKDIPDPALREQIIQQVGQYKGDLERYNKTLVLTGDKIQNLKGLEKLSKLQKLELRQLSNVKEITPELLPESMKKDAELVMVGMTGLEKLNLSGLNRQTLDGIDVNSITHLTSFDISHNSLDLSEKSEDRKLLMTLMEQVSNHQKITVKNTAFENQKPKGYYPQTYDTKEGHYDVDNAEHDILTDFVFGTVTKRNTFIGDEEAFAIYKEGAVDGRQYVSKDYTYEAFRKDYKGYKVHLTASNLGETVTSKVTATTDETYLVDVSDGEKVVHHMKLNIGSGAIMMENLAKGAKVIGTSGDFEQAKKIFDGEKSDRFFTWGQTNWIAFDLGEINLAKEWRLFNAETNTEIKTDSSLNVAKGRLQILKDTTIDLEKMDIKNRKEYLSNDENWTDVAQMDDAKAIFNSKLSNVLSRYWRFCVDGGASSYYPQYTELQILGQRLSNDVANTLD

SEQ ID NO: 8 - protein, 842 aa, Artificial Sequence
  Synthetic
MDKHLLVKRTLGCVCAATLMGAALATHHDSLNTVKAEEKTVQTGKTDQQVGAKLVQEIREGKRGPLYAGYFRTWHDRASTGIDGKQQHPENTMAEVPKEVDILFVFHDHTASDSPFWSELKDSYVHKLHQQGTALVQFIGVNELNGRTGLSKDYPDTPEGNKALAAAIVKAFVTDRGVDGLDIDIEHEFTNKRTPEEDARALNVFKEIAQLIGKNGSDKSKLLIMDTTLSVENNPIFKGIAEDLDYLLRQYYGSQGGEAEVDTINSDWNQYQNYIDASQFMIGFSFFEESASKGNLWFDVNEYDPNNPEKGKDIEGTRAKKYAEWQPSTGGLKAGIFSYAIDRDGVAHVPSTYKNRTSTNLQRHEVDNISHTDYTVSRKLKTLMTEDKRYDVIDQKDIPDPALREQIIQQVGQYKGDLERYNKTLVLTGDKIQNLKGLEKLSKLQKLELRQLSNVKEITPELLPESMKKDAELVMVGMTGLEKLNLSGLNRQTLDGIDVNSITHLTSFDISHNSLDLSEKSEDRKLLMTLMEQVSNHQKITVKNTAFENQKPKGYYPQTYDTKEGHYDVDNAEHDILTDFVFGTVTKRNTFIGDEEAFAIYKEGAVDGRQYVSKDYTYEAFRKDYKGYKVHLTASNLGETVTSKVTATTDETYLVDVSDGEKVVHHMKLNIGSGAIMMENLAKGAKVIGTSGDFEQAKKIFDGEKSDRFFTWGQTNWIAFDLGEINLAKEWRLFNAETNTEIKTDSSLNVAKGRLQILKDTTIDLEKMDIKNRKEYLSNDENWTDVAQMDDAKAIFNSKLSNVLSRYWRFCVDGGASSYYPQYTELQILGQRLSNDVANTLD

SEQ ID NO: 9 - protein, 842 aa, Artificial Sequence
  Synthetic
MDKHLLVKRTLGCVCAATLMGAALATHHDSLNTVKAEEKTVQTGKTDQQVGAKLVQEIREGKRGPLYAGYFRTWHDRASTGIDGKQQHPENTMAEVPKEVDILFVFHDHTASDSPFWSELKDSYVHKLHQQGTALVQHIGVNELNGRTGLSKDYPDTPEGNKALAAAIVKAFVTDRGVDGLDIDIEHEFTNKRTPEEDARALNVFKEIAQLIGKNGSDKSKLLIMDTTLSVENNPIFKGIAEDLDYLLRQYYGSQGGEAEVDTINSDWNQYQNYIDASQFMIGFSFFEESASKGNLWFDVNEYDPNNPEKGKDIEGTRAKKYAEWQPSTGGLKAGIFSYAIDRDGVAHVPSTYKNRTSTNLQRHEVDNISHTDYTVSRKLKTLMTEDKRYDVIDQKDIPDPALREQIIQQVGQYKGDLERYNKTLVLTGDKIQNLKGLEKLSKLQKLELRQLSNVKEITPELLPESMKKDAELVMVGMTGLEKLNLSGLNRQTLDGIDVNSITHLTSFDISHNSLDLSEKSEDRKLLMTLMEQVSNHQKITVKNTAFENQKPKGYYPQTYDTKEGHYDVDNAEHDILTDFVFGTVTKRNTFIGDEEAFAIYKEGAVDGRQYVSKDYTYEAFRKDYKGYKVHLTASNLGETVTSKVTATTDETYLVDVSDGEKVVHHMKLNIGSGAIMMENLAKGAKVIGTSGDFEQAKKIFDGEKSDRFFTWGQTNWIAFDLGEINLAKEWRLFNAETNTEIKTDSSLNVAKGRLQILKDTTIDLEKMDIKNRKEYLSNDENWTDVAQMDDAKAIFNSKLSNVLSRYWRFCVDGGASSYYPQYTELQILGQRLSNDVANTLD

SEQ ID NO: 10 - protein, 842 aa, Artificial Sequence
  Synthetic
MDKHLLVKRTLGCVCAATLMGAALATHHDSLNTVKAEEKTVQTGKTDQQVGAKLVQEIREGKRGPLYAGYFRTWHDRASTGIDGKQQHPENTMAEVPKEVDILFVFHDHTASDSPFWSELKDSYVHKLHQQGTALVQKIGVNELNGRTGLSKDYPDTPEGNKALAAAIVKAFVTDRGVDGLDIDIEHEFTNKRTPEEDARALNVFKEIAQLIGKNGSDKSKLLIMDTTLSVENNPIFKGIAEDLDYLLRQYYGSQGGEAEVDTINSDWNQYQNYIDASQFMIGFSFFEESASKGNLWFDVNEYDPNNPEKGKDIEGTRAKKYAEWQPSTGGLKAGIFSYAIDRDGVAHVPSTYKNRTSTNLQRHEVDNISHTDYTVSRKLKTLMTEDKRYDVIDQKDIPDPALREQIIQQVGQYKGDLERYNKTLVLTGDKIQNLKGLEKLSKLQKLELRQLSNVKEITPELLPESMKKDAELVMVGMTGLEKLNLSGLNRQTLDGIDVNSITHLTSFDISHNSLDLSEKSEDRKLLMTLMEQVSNHQKITVKNTAFENQKPKGYYPQTYDTKEGHYDVDNAEHDILTDFVFGTVTKRNTFIGDEEAFAIYKEGAVDGRQYVSKDYTYEAFRKDYKGYKVHLTASNLGETVTSKVTATTDETYLVDVSDGEKVVHHMKLNIGSGAIMMENLAKGAKVIGTSGDFEQAKKIFDGEKSDRFFTWGQTNWIAFDLGEINLAKEWRLFNAETNTEIKTDSSLNVAKGRLQILKDTTIDLEKMDIKNRKEYLSNDENWTDVAQMDDAKAIFNSKLSNVLSRYWRFCVDGGASSYYPQYTELQILGQRLSNDVANTLD

SEQ ID NO: 11 - protein, 842 aa, Artificial Sequence
  Synthetic
MDKHLLVKRTLGCVCAATLMGAALATHHDSLNTVKAEEKTVQTGKTDQQVGAKLVQEIREGKRGPLYAGYFRTWHDRASTGIDGKQQHPENTMAEVPKEVDILFVFHDHTASDSPFWSELKDSYVHKLHQQGTALVQLIGVNELNGRTGLSKDYPDTPEGNKALAAAIVKAFVTDRGVDGLDIDIEHEFTNKRTPEEDARALNVFKEIAQLIGKNGSDKSKLLIMDTTLSVENNPIFKGIAEDLDYLLRQYYGSQGGEAEVDTINSDWNQYQNYIDASQFMIGFSFFEESASKGNLWFDVNEYDPNNPEKGKDIEGTRAKKYAEWQPSTGGLKAGIFSYAIDRDGVAHVPSTYKNRTSTNLQRHEVDNISHTDYTVSRKLKTLMTEDKRYDVIDQKDIPDPALREQIIQQVGQYKGDLERYNKTLVLTGDKIQNLKGLEKLSKLQKLELRQLSNVKEITPELLPESMKKDAELVMVGMTGLEKLNLSGLNRQTLDGIDVNSITHLTSFDISHNSLDLSEKSEDRKLLMTLMEQVSNHQKITVKNTAFENQKPKGYYPQTYDTKEGHYDVDNAEHDILTDFVFGTVTKRNTFIGDEEAFAIYKEGAVDGRQYVSKDYTYEAFRKDYKGYKVHLTASNLGETVTSKVTATTDETYLVDVSDGEKVVHHMKLNIGSGAIMMENLAKGAKVIGTSGDFEQAKKIFDGEKSDRFFTWGQTNWIAFDLGEINLAKEWRLFNAETNTEIKTDSSLNVAKGRLQILKDTTIDLEKMDIKNRKEYLSNDENWTDVAQMDDAKAIFNSKLSNVLSRYWRFCVDGGASSYYPQYTELQILGQRLSNDVANTLD

SEQ ID NO: 12 - protein, 842 aa, Artificial Sequence
  Synthetic
MDKHLLVKRTLGCVCAATLMGAALATHHDSLNTVKAEEKTVQTGKTDQQVGAKLVQEIREGKRGPLYAGYFRTWHDRASTGIDGKQQHPENTMAEVPKEVDILFVFHDHTASDSPFWSELKDSYVHKLHQQGTALVQMIGVNELNGRTGLSKDYPDTPEGNKALAAAIVKAFVTDRGVDGLDIDIEHEFTNKRTPEEDARALNVFKEIAQLIGKNGSDKSKLLIMDTTLSVENNPIFKGIAEDLDYLLRQYYGSQGGEAEVDTINSDWNQYQNYIDASQFMIGFSFFEESASKGNLWFDVNEYDPNNPEKGKDIEGTRAKKYAEWQPSTGGLKAGIFSYAIDRDGVAHVPSTYKNRTSTNLQRHEVDNISHTDYTVSRKLKTLMTEDKRYDVIDQKDIPDPALREQIIQQVGQYKGDLERYNKTLVLTGDKIQNLKGLEKLSKLQKLELRQLSNVKEITPELLPESMKKDAELVMVGMTGLEKLNLSGLNRQTLDGIDVNSITHLTSFDISHNSLDLSEKSEDRKLLMTLMEQVSNHQKITVKNTAFENQKPKGYYPQTYDTKEGHYDVDNAEHDILTDFVFGTVTKRNTFIGDEEAFAIYKEGAVDGRQYVSKDYTYEAFRKDYKGYKVHLTASNLGETVTSKVTATTDETYLVDVSDGEKVVHHMKLNIGSGAIMMENLAKGAKVIGTSGDFEQAKKIFDGEKSDRFFTWGQTNWIAFDLGEINLAKEWRLFNAETNTEIKTDSSLNVAKGRLQILKDTTIDLEKMDIKNRKEYLSNDENWTDVAQMDDAKAIFNSKLSNVLSRYWRFCVDGGASSYYPQYTELQILGQRLSNDVANTLD

SEQ ID NO: 13 - protein, 842 aa, Artificial Sequence
  Synthetic
MDKHLLVKRTLGCVCAATLMGAALATHHDSLNTVKAEEKTVQTGKTDQQVGAKLVQEIREGKRGPLYAGYFRTWHDRASTGIDGKQQHPENTMAEVPKEVDILFVFHDHTASDSPFWSELKDSYVHKLHQQGTALVQNIGVNELNGRTGLSKDYPDTPEGNKALAAAIVKAFVTDRGVDGLDIDIEHEFTNKRTPEEDARALNVFKEIAQLIGKNGSDKSKLLIMDTTLSVENNPIFKGIAEDLDYLLRQYYGSQGGEAEVDTINSDWNQYQNYIDASQFMIGFSFFEESASKGNLWFDVNEYDPNNPEKGKDIEGTRAKKYAEWQPSTGGLKAGIFSYAIDRDGVAHVPSTYKNRTSTNLQRHEVDNISHTDYTVSRKLKTLMTEDKRYDVIDQKDIPDPALREQIIQQVGQYKGDLERYNKTLVLTGDKIQNLKGLEKLSKLQKLELRQLSNVKEITPELLPESMKKDAELVMVGMTGLEKLNLSGLNRQTLDGIDVNSITHLTSFDISHNSLDLSEKSEDRKLLMTLMEQVSNHQKITVKNTAFENQKPKGYYPQTYDTKEGHYDVDNAEHDILTDFVFGTVTKRNTFIGDEEAFAIYKEGAVDGRQYVSKDYTYEAFRKDYKGYKVHLTASNLGETVTSKVTATTDETYLVDVSDGEKVVHHMKLNIGSGAIMMENLAKGAKVIGTSGDFEQAKKIFDGEKSDRFFTWGQTNWIAFDLGEINLAKEWRLFNAETNTEIKTDSSLNVAKGRLQILKDTTIDLEKMDIKNRKEYLSNDENWTDVAQMDDAKAIFNSKLSNVLSRYWRFCVDGGASSYYPQYTELQILGQRLSNDVANTLD

SEQ ID NO: 14 - protein, 842 aa, Artificial Sequence
  Synthetic
MDKHLLVKRTLGCVCAATLMGAALATHHDSLNTVKAEEKTVQTGKTDQQVGAKLVQEIREGKRGPLYAGYFRTWHDRASTGIDGKQQHPENTMAEVPKEVDILFVFHDHTASDSPFWSELKDSYVHKLHQQGTALVQQIGVNELNGRTGLSKDYPDTPEGNKALAAAIVKAFVTDRGVDGLDIDIEHEFTNKRTPEEDARALNVFKEIAQLIGKNGSDKSKLLIMDTTLSVENNPIFKGIAEDLDYLLRQYYGSQGGEAEVDTINSDWNQYQNYIDASQFMIGFSFFEESASKGNLWFDVNEYDPNNPEKGKDIEGTRAKKYAEWQPSTGGLKAGIFSYAIDRDGVAHVPSTYKNRTSTNLQRHEVDNISHTDYTVSRKLKTLMTEDKRYDVIDQKDIPDPALREQIIQQVGQYKGDLERYNKTLVLTGDKIQNLKGLEKLSKLQKLELRQLSNVKEITPELLPESMKKDAELVMVGMTGLEKLNLSGLNRQTLDGIDVNSITHLTSFDISHNSLDLSEKSEDRKLLMTLMEQVSNHQKITVKNTAFENQKPKGYYPQTYDTKEGHYDVDNAEHDILTDFVFGTVTKRNTFIGDEEAFAIYKEGAVDGRQYVSKDYTYEAFRKDYKGYKVHLTASNLGETVTSKVTATTDETYLVDVSDGEKVVHHMKLNIGSGAIMMENLAKGAKVIGTSGDFEQAKKIFDGEKSDRFFTWGQTNWIAFDLGEINLAKEWRLFNAETNTEIKTDSSLNVAKGRLQILKDTTIDLEKMDIKNRKEYLSNDENWTDVAQMDDAKAIFNSKLSNVLSRYWRFCVDGGASSYYPQYTELQILGQRLSNDVANTLD

SEQ ID NO: 15 - protein, 842 aa, Artificial Sequence
  Synthetic
MDKHLLVKRTLGCVCAATLMGAALATHHDSLNTVKAEEKTVQTGKTDQQVGAKLVQEIREGKRGPLYAGYFRTWHDRASTGIDGKQQHPENTMAEVPKEVDILFVFHDHTASDSPFWSELKDSYVHKLHQQGTALVQRIGVNELNGRTGLSKDYPDTPEGNKALAAAIVKAFVTDRGVDGLDIDIEHEFTNKRTPEEDARALNVFKEIAQLIGKNGSDKSKLLIMDTTLSVENNPIFKGIAEDLDYLLRQYYGSQGGEAEVDTINSDWNQYQNYIDASQFMIGFSFFEESASKGNLWFDVNEYDPNNPEKGKDIEGTRAKKYAEWQPSTGGLKAGIFSYAIDRDGVAHVPSTYKNRTSTNLQRHEVDNISHTDYTVSRKLKTLMTEDKRYDVIDQKDIPDPALREQIIQQVGQYKGDLERYNKTLVLTGDKIQNLKGLEKLSKLQKLELRQLSNVKEITPELLPESMKKDAELVMVGMTGLEKLNLSGLNRQTLDGIDVNSITHLTSFDISHNSLDLSEKSEDRKLLMTLMEQVSNHQKITVKNTAFENQKPKGYYPQTYDTKEGHYDVDNAEHDILTDFVFGTVTKRNTFIGDEEAFAIYKEGAVDGRQYVSKDYTYEAFRKDYKGYKVHLTASNLGETVTSKVTATTDETYLVDVSDGEKVVHHMKLNIGSGAIMMENLAKGAKVIGTSGDFEQAKKIFDGEKSDRFFTWGQTNWIAFDLGEINLAKEWRLFNAETNTEIKTDSSLNVAKGRLQILKDTTIDLEKMDIKNRKEYLSNDENWTDVAQMDDAKAIFNSKLSNVLSRYWRFCVDGGASSYYPQYTELQILGQRLSNDVANTLD

SEQ ID NO: 16 - protein, 842 aa, Artificial Sequence
  Synthetic
MDKHLLVKRTLGCVCAATLMGAALATHHDSLNTVKAEEKTVQTGKTDQQVGAKLVQEIREGKRGPLYAGYFRTWHDRASTGIDGKQQHPENTMAEVPKEVDILFVFHDHTASDSPFWSELKDSYVHKLHQQGTALVQVIGVNELNGRTGLSKDYPDTPEGNKALAAAIVKAFVTDRGVDGLDIDIEHEFTNKRTPEEDARALNVFKEIAQLIGKNGSDKSKLLIMDTTLSVENNPIFKGIAEDLDYLLRQYYGSQGGEAEVDTINSDWNQYQNYIDASQFMIGFSFFEESASKGNLWFDVNEYDPNNPEKGKDIEGTRAKKYAEWQPSTGGLKAGIFSYAIDRDGVAHVPSTYKNRTSTNLQRHEVDNISHTDYTVSRKLKTLMTEDKRYDVIDQKDIPDPALREQIIQQVGQYKGDLERYNKTLVLTGDKIQNLKGLEKLSKLQKLELRQLSNVKEITPELLPESMKKDAELVMVGMTGLEKLNLSGLNRQTLDGIDVNSITHLTSFDISHNSLDLSEKSEDRKLLMTLMEQVSNHQKITVKNTAFENQKPKGYYPQTYDTKEGHYDVDNAEHDILTDFVFGTVTKRNTFIGDEEAFAIYKEGAVDGRQYVSKDYTYEAFRKDYKGYKVHLTASNLGETVTSKVTATTDETYLVDVSDGEKVVHHMKLNIGSGAIMMENLAKGAKVIGTSGDFEQAKKIFDGEKSDRFFTWGQTNWIAFDLGEINLAKEWRLFNAETNTEIKTDSSLNVAKGRLQILKDTTIDLEKMDIKNRKEYLSNDENWTDVAQMDDAKAIFNSKLSNVLSRYWRFCVDGGASSYYPQYTELQILGQRLSNDVANTLD

SEQ ID NO: 17 - protein, 842 aa, Artificial Sequence
  Synthetic
MDKHLLVKRTLGCVCAATLMGAALATHHDSLNTVKAEEKTVQTGKTDQQVGAKLVQEIREGKRGPLYAGYFRTWHDRASTGIDGKQQHPENTMAEVPKEVDILFVFHDHTASDSPFWSELKDSYVHKLHQQGTALVQWIGVNELNGRTGLSKDYPDTPEGNKALAAAIVKAFVTDRGVDGLDIDIEHEFTNKRTPEEDARALNVFKEIAQLIGKNGSDKSKLLIMDTTLSVENNPIFKGIAEDLDYLLRQYYGSQGGEAEVDTINSDWNQYQNYIDASQFMIGFSFFEESASKGNLWFDVNEYDPNNPEKGKDIEGTRAKKYAEWQPSTGGLKAGIFSYAIDRDGVAHVPSTYKNRTSTNLQRHEVDNISHTDYTVSRKLKTLMTEDKRYDVIDQKDIPDPALREQIIQQVGQYKGDLERYNKTLVLTGDKIQNLKGLEKLSKLQKLELRQLSNVKEITPELLPESMKKDAELVMVGMTGLEKLNLSGLNRQTLDGIDVNSITHLTSFDISHNSLDLSEKSEDRKLLMTLMEQVSNHQKITVKNTAFENQKPKGYYPQTYDTKEGHYDVDNAEHDILTDFVFGTVTKRNTFIGDEEAFAIYKEGAVDGRQYVSKDYTYEAFRKDYKGYKVHLTASNLGETVTSKVTATTDETYLVDVSDGEKVVHHMKLNIGSGAIMMENLAKGAKVIGTSGDFEQAKKIFDGEKSDRFFTWGQTNWIAFDLGEINLAKEWRLFNAETNTEIKTDSSLNVAKGRLQILKDTTIDLEKMDIKNRKEYLSNDENWTDVAQMDDAKAIFNSKLSNVLSRYWRFCVDGGASSYYPQYTELQILGQRLSNDVANTLD

SEQ ID NO: 18 - protein, 451 aa, Artificial Sequence
  Synthetic
QVQLQQPGAELVKPGASVKMSCKASGYTFTSYNMHWVKQTPGRGLEWIGAIYPGNGDTSYNQKFKGKATLTADKSSSTAYMQLSSLTSEDSAVYYCARSTYYGGDWYFNVWGAGTTVTVSAASTKGPSVFPLAPSSKSTSGGTAALGCLVKDYFPEPVTVSWNSGALTSGVHTFPAVLQSSGLYSLSSVVTVPSSSLGTQTYICNVNHKPSNTKVDKKVEPKSCDKTHTCPPCPAPELLGGPSVFLFPPKPKDTLMISRTPEVTCVVVDVSHEDPEVKFNWYVDGVEVHNAKTKPREEQYNSTYRVVSVLTVLHQDWLNGKEYKCKVSNKALPAPIEKTISKAKGQPREPQVYTLPPSRDELTKNQVSLTCLVKGFYPSDIAVEWESNGQPENNYKTTPPVLDSDGSFFLYSKLTVDKSRWQQGNVFSCSVMHEALHNHYTQKSLSLSPGK

SEQ ID NO: 19 - protein, 212 aa, Artificial Sequence
  Synthetic
QIVLSQSPAILSASPGEKVTMTCRASSSVSYIHWFQQKPGSSPKPWIYATNLASGVPVRFSGSGSGTSYSLTISRVEAEDAATYYCQQWTSNPPTFGGGTKLEIKRTVAAPSVFIFPPSDEQLKSGTASVVCLLNNFYPREAKVQWKVDNALQSGNSQESVTEQDSKDSTYSLSSTLTLSKADYEKHKVYACEVTHQGLSSPVTKSFNRGEC